European Patent Specification EP 3 515 489 B1, published November 5, 2025. Title: CD80 and CD86 binding protein compositions and uses thereof. Applicant: OncoImmune, Inc. Children's Research Institute, Children's National Medical Center Liu, Yang Devenport, Martin Zheng, Pan Wu, Wei Du, Xuexiang Liu, Mingyue Tang, Fei. The sequence listing filed with the application follows.

SEQUENCE LISTING (50 sequences)

SEQ ID NO: 1 - protein, 223 aa, Homo sapiens
MACLGFQRHKAQLNLATRTWPCTLLFFLLFIPVFCKAMHVAQPAVVLASSRGIASFVCEYASPGKATEVRVTVLRQADSQVTEVCAATYMMGNELTFLDDSICTGTSSGNQVNLTIQGLRAMDTGLYICKVELMYPPPYYLGIGNGTQIYVIDPEPCPDSDFLLWILAAVSSGLFFYSFLLTAVSLSKMLKKRSPLTTGVYVKMPPTEPECEKQFQPYFIPIN

SEQ ID NO: 2 - protein, 357 aa, Homo sapiens [sequence omitted]

SEQ ID NO: 3 - protein, 126 aa, Homo sapiens [sequence omitted]

SEQ ID NO: 4 - protein, 174 aa, Homo sapiens
MACLGFQRHKAQLNLATRTWPCTLLFFLLFIPVFCKAMHVAQPAVVLASSRGIASFVCEYASPGKATEVRVTVLRQADSQVTEVCAATYMMGNELTFLDDSICTGTSSGNQVNLTIQGLRAMDTGLYICKVELMYPPPYYLGIGNGTQIYVIAKEKKPSYNRGLCENAPNRARM

SEQ ID NO: 5 - protein, 223 aa, Mus musculus
MACLGLRRYKAQLQLPSRTWPFVALLTLLFIPVFSEAIQVTQPSVVLASSHGVASFPCEYSPSHNTDEVRVTVLRQTNDQMTEVCATTFTEKNTVGFLDYPFCSGTFNESRVNLTIQGLRAVDTGLYLCKVELMYPPPYFVGMGNGTQIYVIDPEPCPDSDFLLWILVAVSLGLFFYSFLVSAVSLSKMLKKRSPLTTGVYVKMPPTEPECEKQFQPYFIPIN

SEQ ID NO: 6 - protein, 126 aa, Mus musculus
EAIQVTQPSVVLASSHGVASFPCEYSPSHNTDEVRVTVLRQTNDQMTEVCATTFTEKNTVGFLDYPFCSGTFNESRVNLTIQGLRAVDTGLYLCKVELMYPPPYFVGMGNGTQIYVIDPEPCPDSD

SEQ ID NO: 7 - protein, 357 aa, Artificial Sequence
  Fusion protein
IQVTQPSVVLASSRGIASFVCEYASPGKATEVRVTVLRQADSQVTEVCAATYMMGNELTFLDDSICTGTSSGNQVNLTIQGLRAMDTGLYICKVELMYPPPYYLGIGNGTQIYVIDPEPCPDSDQEPKSSDKTHTSPPSPAPELLGGSSVFLFPPKPKDTLMISRTPEVTCVVVDVSHEDPEVKFNWYVDGVEVHNAKTKPREEQYNSTYRVVSVLTVLHQDWLNGKEYKCKVSNKALPAPIEKTISKAKGQPREPQVYTLPPSRDELTKNQVSLTCLVKGFYPSDIAVEWESNGQPENNYKTTPPVLDSDGSFFLYSKLTVDKSRWQQGNVFSCSVMHEALHNHYTQKSLSLSPGK

SEQ ID NO: 8 - protein, 357 aa, Artificial Sequence
  Fusion protein
MHVAQPAVVLASSHGLASFPCEYASPGKATEVRVTVLRQADSQVTEVCAATYMMGNELTFLDDSICTGTSSGNQVNLTIQGLRAMDTGLYICKVELMYPPPYYLGIGNGTQIYVIDPEPCPDSDQEPKSSDKTHTSPPSPAPELLGGSSVFLFPPKPKDTLMISRTPEVTCVVVDVSHEDPEVKFNWYVDGVEVHNAKTKPREEQYNSTYRVVSVLTVLHQDWLNGKEYKCKVSNKALPAPIEKTISKAKGQPREPQVYTLPPSRDELTKNQVSLTCLVKGFYPSDIAVEWESNGQPENNYKTTPPVLDSDGSFFLYSKLTVDKSRWQQGNVFSCSVMHEALHNHYTQKSLSLSPGK

SEQ ID NO: 9 - protein, 358 aa, Artificial Sequence
  Fusion protein
MHVAQPAVVLASSRGIASFVCEYASPSHNTDEVRVTVLRQADSQVTEVCAATYMMGNELTFLDDSICTGTSSGNQVNLTIQGLRAMDTGLYICKVELMYPPPYYLGIGNGTQIYVIDPEPCPDSDQEPKSSDKTHTSPPSPAPELLGGSSVFLFPPKPKDTLMISRTPEVTCVVVDVSHEDPEVKFNWYVDGVEVHNAKTKPREEQYNSTYRVVSVLTVLHQDWLNGKEYKCKVSNKALPAPIEKTISKAKGQPREPQVYTLPPSRDELTKNQVSLTCLVKGFYPSDIAVEWESNGQPENNYKTTPPVLDSDGSFFLYSKLTVDKSRWQQGNVFSCSVMHEALHNHYTQKSLSLSPGK

SEQ ID NO: 10 - protein, 357 aa, Artificial Sequence
  Fusion protein
MHVAQPAVVLASSRGIASFVCEYASPGKATEVRVTVLRTNDQMVTEVCAATYMMGNELTFLDDSICTGTSSGNQVNLTIQGLRAMDTGLYICKVELMYPPPYYLGIGNGTQIYVIDPEPCPDSDQEPKSSDKTHTSPPSPAPELLGGSSVFLFPPKPKDTLMISRTPEVTCVVVDVSHEDPEVKFNWYVDGVEVHNAKTKPREEQYNSTYRVVSVLTVLHQDWLNGKEYKCKVSNKALPAPIEKTISKAKGQPREPQVYTLPPSRDELTKNQVSLTCLVKGFYPSDIAVEWESNGQPENNYKTTPPVLDSDGSFFLYSKLTVDKSRWQQGNVFSCSVMHEALHNHYTQKSLSLSPGK

SEQ ID NO: 11 - protein, 357 aa, Artificial Sequence
  Fusion protein
MHVAQPAVVLASSRGIASFVCEYASPGKATEVRVTVLRQADSQVTEVCAATFTEKNTVGFLDDSICTGTSSGNQVNLTIQGLRAMDTGLYICKVELMYPPPYYLGIGNGTQIYVIDPEPCPDSDQEPKSSDKTHTSPPSPAPELLGGSSVFLFPPKPKDTLMISRTPEVTCVVVDVSHEDPEVKFNWYVDGVEVHNAKTKPREEQYNSTYRVVSVLTVLHQDWLNGKEYKCKVSNKALPAPIEKTISKAKGQPREPQVYTLPPSRDELTKNQVSLTCLVKGFYPSDIAVEWESNGQPENNYKTTPPVLDSDGSFFLYSKLTVDKSRWQQGNVFSCSVMHEALHNHYTQKSLSLSPGK

SEQ ID NO: 12 - protein, 357 aa, Artificial Sequence
  Fusion protein
MHVAQPAVVLASSRGIASFVCEYASPGKATEVRVTVLRQADSQVTEVCATTYMMGNELTFLDDSICTGTSSGNQVNLTIQGLRAMDTGLYICKVELMYPPPYYLGIGNGTQIYVIDPEPCPDSDQEPKSSDKTHTSPPSPAPELLGGSSVFLFPPKPKDTLMISRTPEVTCVVVDVSHEDPEVKFNWYVDGVEVHNAKTKPREEQYNSTYRVVSVLTVLHQDWLNGKEYKCKVSNKALPAPIEKTISKAKGQPREPQVYTLPPSRDELTKNQVSLTCLVKGFYPSDIAVEWESNGQPENNYKTTPPVLDSDGSFFLYSKLTVDKSRWQQGNVFSCSVMHEALHNHYTQKSLSLSPGK

SEQ ID NO: 13 - protein, 357 aa, Artificial Sequence
  Fusion protein
MHVAQPAVVLASSRGIASFVCEYASPGKATEVRVTVLRQADSQVTEVCAATYMMGNELTFLDYPFCSGTSSGNQVNLTIQGLRAMDTGLYICKVELMYPPPYYLGIGNGTQIYVIDPEPCPDSDQEPKSSDKTHTSPPSPAPELLGGSSVFLFPPKPKDTLMISRTPEVTCVVVDVSHEDPEVKFNWYVDGVEVHNAKTKPREEQYNSTYRVVSVLTVLHQDWLNGKEYKCKVSNKALPAPIEKTISKAKGQPREPQVYTLPPSRDELTKNQVSLTCLVKGFYPSDIAVEWESNGQPENNYKTTPPVLDSDGSFFLYSKLTVDKSRWQQGNVFSCSVMHEALHNHYTQKSLSLSPGK

SEQ ID NO: 14 - protein, 357 aa, Artificial Sequence
  Fusion protein
MHVAQPAVVLASSRGIASFVCEYASPGKATEVRVTVLRQADSQVTEVCAATYMMGNELTFLDDSICTGTFNESRVNLTIQGLRAMDTGLYICKVELMYPPPYYLGIGNGTQIYVIDPEPCPDSDQEPKSSDKTHTSPPSPAPELLGGSSVFLFPPKPKDTLMISRTPEVTCVVVDVSHEDPEVKFNWYVDGVEVHNAKTKPREEQYNSTYRVVSVLTVLHQDWLNGKEYKCKVSNKALPAPIEKTISKAKGQPREPQVYTLPPSRDELTKNQVSLTCLVKGFYPSDIAVEWESNGQPENNYKTTPPVLDSDGSFFLYSKLTVDKSRWQQGNVFSCSVMHEALHNHYTQKSLSLSPGK

SEQ ID NO: 15 - protein, 358 aa, Artificial Sequence
  Fusion protein
MHVAQPAVVLASSRGIASFVCEYASPGKATEVRVTVLRQADSQVTEVCAATYMMGNELTFLDDSICTGTSSGNQVNLTIQGLRAMVDTGLYICKVELMYPPPYYLGIGNGTQIYVIDPEPCPDSDQEPKSSDKTHTSPPSPAPELLGGSSVFLFPPKPKDTLMISRTPEVTCVVVDVSHEDPEVKFNWYVDGVEVHNAKTKPREEQYNSTYRVVSVLTVLHQDWLNGKEYKCKVSNKALPAPIEKTISKAKGQPREPQVYTLPPSRDELTKNQVSLTCLVKGFYPSDIAVEWESNGQPENNYKTTPPVLDSDGSFFLYSKLTVDKSRWQQGNVFSCSVMHEALHNHYTQKSLSLSPGK

SEQ ID NO: 16 - protein, 358 aa, Artificial Sequence
  Fusion protein
MHVAQPAVVLASSRGIASFVCEYASPGKATEVRVTVLRQADSQVTEVCAATYMMGNELTFLDDSICTGTSSGNQVNLTIQGLRAMMDTGLYLCKVELMYPPPYYLGIGNGTQIYVIDPEPCPDSDQEPKSSDKTHTSPPSPAPELLGGSSVFLFPPKPKDTLMISRTPEVTCVVVDVSHEDPEVKFNWYVDGVEVHNAKTKPREEQYNSTYRVVSVLTVLHQDWLNGKEYKCKVSNKALPAPIEKTISKAKGQPREPQVYTLPPSRDELTKNQVSLTCLVKGFYPSDIAVEWESNGQPENNYKTTPPVLDSDGSFFLYSKLTVDKSRWQQGNVFSCSVMHEALHNHYTQKSLSLSPGK

SEQ ID NO: 17 - protein, 357 aa, artificial
  Fusion protein
MHVAQPAVVLASSRGIASFVCEYASPGKATEVRVTVLRQADSQVTEVCAATYMMGNELTFLDDSICTGTSSGNQVNLTIQGLRAMDTGLYICKVELMYPPPYFVGMGNGTQIYVIDPEPCPDSDQEPKSSDKTHTSPPSPAPELLGGSSVFLFPPKPKDTLMISRTPEVTCVVVDVSHEDPEVKFNWYVDGVEVHNAKTKPREEQYNSTYRVVSVLTVLHQDWLNGKEYKCKVSNKALPAPIEKTISKAKGQPREPQVYTLPPSRDELTKNQVSLTCLVKGFYPSDIAVEWESNGQPENNYKTTPPVLDSDGSFFLYSKLTVDKSRWQQGNVFSCSVMHEALHNHYTQKSLSLSPGK

SEQ ID NO: 18 - protein, 357 aa, artificial
  Fusion protein
IQVTQPSVVLASSRGIASFVCEYASPGKATEVRVTVLRQADSQVTEVCAATFTEKNTVGFLDDSICTGTFNESRVNLTIQGLRAMDTGLYICKVELMYPPPYFVGMGNGTQIYVIDPEPCPDSDQEPKSSDKTHTSPPSPAPELLGGSSVFLFPPKPKDTLMISRTPEVTCVVVDVSHEDPEVKFNWYVDGVEVHNAKTKPREEQYNSTYRVVSVLTVLHQDWLNGKEYKCKVSNKALPAPIEKTISKAKGQPREPQVYTLPPSRDELTKNQVSLTCLVKGFYPSDIAVEWESNGQPENNYKTTPPVLDSDGSFFLYSKLTVDKSRWQQGNVFSCSVMHEALHNHYTQKSLSLSPGK

SEQ ID NO: 19 - protein, 357 aa, artificial
  Fusion protein
MHVAQPAVVLASSRGIASFVCEYASPGKYTEVRVTVLRQADSQVTEVCAATYMMGNELTFLDDSICTGTSSGNQVNLTIQGLRAMDTGLYICKVELMYPPPYFVGMGNGTQIYVIDPEPCPDSDQEPKSSDKTHTSPPSPAPELLGGSSVFLFPPKPKDTLMISRTPEVTCVVVDVSHEDPEVKFNWYVDGVEVHNAKTKPREEQYNSTYRVVSVLTVLHQDWLNGKEYKCKVSNKALPAPIEKTISKAKGQPREPQVYTLPPSRDELTKNQVSLTCLVKGFYPSDIAVEWESNGQPENNYKTTPPVLDSDGSFFLYSKLTVDKSRWQQGNVFSCSVMHEALHNHYTQKSLSLSPGK

SEQ ID NO: 20 - protein, 357 aa, Artificial Sequence
  Fusion protein
IQVTQPSVVLASSRGIASFVCEYASPGKATEVRVTVLRQADSQVTEVCAATFTEKNTVGFLDDSICTGTSSGNQVNLTIQGLRAMDTGLYICKVELMYPPPYFVGMGNGTQIYVIDPEPCPDSDQEPKSSDKTHTSPPSPAPELLGGSSVFLFPPKPKDTLMISRTPEVTCVVVDVSHEDPEVKFNWYVDGVEVHNAKTKPREEQYNSTYRVVSVLTVLHQDWLNGKEYKCKVSNKALPAPIEKTISKAKGQPREPQVYTLPPSRDELTKNQVSLTCLVKGFYPSDIAVEWESNGQPENNYKTTPPVLDSDGSFFLYSKLTVDKSRWQQGNVFSCSVMHEALHNHYTQKSLSLSPGK

SEQ ID NO: 21 - protein, 357 aa, Artificial Sequence
  Fusion protein
MHVAQPAVVLASSRGIASFVCEYASPGKYTEVRVTVLRQADSQVTEVCAATYMMGNELTFLDDSICTGTSSGNQVNLTIQGLRAMDTGLYICKVELMYPPPYYEGIGNGTQIYVIDPEPCPDSDQEPKSSDKTHTSPPSPAPELLGGSSVFLFPPKPKDTLMISRTPEVTCVVVDVSHEDPEVKFNWYVDGVEVHNAKTKPREEQYNSTYRVVSVLTVLHQDWLNGKEYKCKVSNKALPAPIEKTISKAKGQPREPQVYTLPPSRDELTKNQVSLTCLVKGFYPSDIAVEWESNGQPENNYKTTPPVLDSDGSFFLYSKLTVDKSRWQQGNVFSCSVMHEALHNHYTQKSLSLSPGK

SEQ ID NO: 22 - protein, 357 aa, Artificial Sequence
  Fusion protein
IQVTQPSVVLASSRGIASFVCEYASPGKATEVRVTVLRQADSQVTEVCAATFTEKNTVGFLDDSICTGTFNESRVNLTIQGLRAMDTGLYICKVELMYPPPYFVGMGNGTQIYVIDPEPCPDSDQEPKSSDKTHTSPPSPAPELLGGSSVFLFPPKPKDTLYITREPEVTCVVVDVSHEDPEVKFNWYVDGVEVHNAKTKPREEQYNSTYRVVSVLTVLHQDWLNGKEYKCKVSNKALPAPIEKTISKAKGQPREPQVYTLPPSRDELTKNQVSLTCLVKGFYPSDIAVEWESNGQPENNYKTTPPVLDSDGSFFLYSKLTVDKSRWQQGNVFSCSVMHEALHNHYTQKSLSLSPGK

SEQ ID NO: 23 - protein, 357 aa, Artificial Sequence
  Fusion protein
MHVAQPAVVLASSRGIASFVCEYASPGKYTEVRVTVLRQADSQVTEVCAATYMMGNELTFLDDSICTGTSSGNQVNLTIQGLRAMDTGLYICKVELMYPPPYFEGMGNGTQIYVIDPEPCPDSDQEPKSSDKTHTSPPSPAPELLGGSSVFLFPPKPKDTLMISRTPEVTCVVVDVSHEDPEVKFNWYVDGVEVHNAKTKPREEQYNSTYRVVSVLTVLHQDWLNGKEYKCKVSNKALPAPIEKTISKAKGQPREPQVYTLPPSRDELTKNQVSLTCLVKGFYPSDIAVEWESNGQPENNYKTTPPVLDSDGSFFLYSKLTVDKSRWQQGNVFSCSVMHEALHNHYTQKSLSLSPGK

SEQ ID NO: 24 - protein, 124 aa, Artificial Sequence
  Mutant
IQVTQPSVVLASSRGIASFVCEYASPGKATEVRVTVLRQADSQVTEVCAATYMMGNELTFLDDSICTGTSSGNQVNLTIQGLRAMDTGLYICKVELMYPPPYYLGIGNGTQIYVIDPEPCPDSD

SEQ ID NO: 25 - protein, 124 aa, Artificial Sequence
  Mutant
MHVAQPAVVLASSHGLASFPCEYASPGKATEVRVTVLRQADSQVTEVCAATYMMGNELTFLDDSICTGTSSGNQVNLTIQGLRAMDTGLYICKVELMYPPPYYLGIGNGTQIYVIDPEPCPDSD

SEQ ID NO: 26 - protein, 125 aa, Artificial Sequence
  Mutant
MHVAQPAVVLASSRGIASFVCEYASPSHNTDEVRVTVLRQADSQVTEVCAATYMMGNELTFLDDSICTGTSSGNQVNLTIQGLRAMDTGLYICKVELMYPPPYYLGIGNGTQIYVIDPEPCPDSD

SEQ ID NO: 27 - protein, 124 aa, Artificial Sequence
  Mutant
MHVAQPAVVLASSRGIASFVCEYASPGKATEVRVTVLRTNDQMVTEVCAATYMMGNELTFLDDSICTGTSSGNQVNLTIQGLRAMDTGLYICKVELMYPPPYYLGIGNGTQIYVIDPEPCPDSD

SEQ ID NO: 28 - protein, 124 aa, Artificial Sequence
  Mutant
MHVAQPAVVLASSRGIASFVCEYASPGKATEVRVTVLRQADSQVTEVCAATFTEKNTVGFLDDSICTGTSSGNQVNLTIQGLRAMDTGLYICKVELMYPPPYYLGIGNGTQIYVIDPEPCPDSD

SEQ ID NO: 29 - protein, 124 aa, Artificial Sequence
  Mutant
MHVAQPAVVLASSRGIASFVCEYASPGKATEVRVTVLRQADSQVTEVCATTYMMGNELTFLDDSICTGTSSGNQVNLTIQGLRAMDTGLYICKVELMYPPPYYLGIGNGTQIYVIDPEPCPDSD

SEQ ID NO: 30 - protein, 124 aa, Artificial
  Mutant
MHVAQPAVVLASSRGIASFVCEYASPGKATEVRVTVLRQADSQVTEVCAATYMMGNELTFLDYPFCSGTSSGNQVNLTIQGLRAMDTGLYICKVELMYPPPYYLGIGNGTQIYVIDPEPCPDSD

SEQ ID NO: 31 - protein, 124 aa, Artificial Sequence
  Mutant
MHVAQPAVVLASSRGIASFVCEYASPGKATEVRVTVLRQADSQVTEVCAATYMMGNELTFLDDSICTGTFNESRVNLTIQGLRAMDTGLYICKVELMYPPPYYLGIGNGTQIYVIDPEPCPDSD

SEQ ID NO: 32 - protein, 125 aa, Artificial Sequence
  Mutant
MHVAQPAVVLASSRGIASFVCEYASPGKATEVRVTVLRQADSQVTEVCAATYMMGNELTFLDDSICTGTSSGNQVNLTIQGLRAMVDTGLYICKVELMYPPPYYLGIGNGTQIYVIDPEPCPDSD

SEQ ID NO: 33 - protein, 125 aa, Artificial
  Mutant
MHVAQPAVVLASSRGIASFVCEYASPGKATEVRVTVLRQADSQVTEVCAATYMMGNELTFLDDSICTGTSSGNQVNLTIQGLRAMMDTGLYLCKVELMYPPPYYLGIGNGTQIYVIDPEPCPDSD

SEQ ID NO: 34 - protein, 124 aa, Artificial Sequence
  Mutant
MHVAQPAVVLASSRGIASFVCEYASPGKATEVRVTVLRQADSQVTEVCAATYMMGNELTFLDDSICTGTSSGNQVNLTIQGLRAMDTGLYICKVELMYPPPYFVGMGNGTQIYVIDPEPCPDSD

SEQ ID NO: 35 - protein, 124 aa, Artificial Sequence
  Mutant
IQVTQPSVVLASSRGIASFVCEYASPGKATEVRVTVLRQADSQVTEVCAATFTEKNTVGFLDDSICTGTFNESRVNLTIQGLRAMDTGLYICKVELMYPPPYFVGMGNGTQIYVIDPEPCPDSD

SEQ ID NO: 36 - protein, 124 aa, Artificial Sequence
  Mutant
MHVAQPAVVLASSRGIASFVCEYASPGKYTEVRVTVLRQADSQVTEVCAATYMMGNELTFLDDSICTGTSSGNQVNLTIQGLRAMDTGLYICKVELMYPPPYFVGMGNGTQIYVIDPEPCPDSD

SEQ ID NO: 37 - protein, 124 aa, Artificial Sequence
  Mutant
IQVTQPSVVLASSRGIASFVCEYASPGKATEVRVTVLRQADSQVTEVCAATFTEKNTVGFLDDSICTGTSSGNQVNLTIQGLRAMDTGLYICKVELMYPPPYFVGMGNGTQIYVIDPEPCPDSD

SEQ ID NO: 38 - protein, 124 aa, Artificial Sequence
  Mutant
MHVAQPAVVLASSRGIASFVCEYASPGKYTEVRVTVLRQADSQVTEVCAATYMMGNELTFLDDSICTGTSSGNQVNLTIQGLRAMDTGLYICKVELMYPPPYYEGIGNGTQIYVIDPEPCPDSD

SEQ ID NO: 39 - protein, 124 aa, Artificial Sequence; identical to SEQ ID NO: 35
  Mutant

SEQ ID NO: 40 - protein, 124 aa, Artificial Sequence
  Mutant
MHVAQPAVVLASSRGIASFVCEYASPGKYTEVRVTVLRQADSQVTEVCAATYMMGNELTFLDDSICTGTSSGNQVNLTIQGLRAMDTGLYICKVELMYPPPYFEGMGNGTQIYVIDPEPCPDSD

SEQ ID NO: 41 - protein, 233 aa, Homo sapiens
QEPKSSDKTHTSPPSPAPELLGGSSVFLFPPKPKDTLMISRTPEVTCVVVDVSHEDPEVKFNWYVDGVEVHNAKTKPREEQYNSTYRVVSVLTVLHQDWLNGKEYKCKVSNKALPAPIEKTISKAKGQPREPQVYTLPPSRDELTKNQVSLTCLVKGFYPSDIAVEWESNGQPENNYKTTPPVLDSDGSFFLYSKLTVDKSRWQQGNVFSCSVMHEALHNHYTQKSLSLSPGK

SEQ ID NO: 42 - protein, 357 aa, Artificial Sequence; identical to SEQ ID NO: 19
  Fusion protein

SEQ ID NO: 43 - protein, 357 aa, Artificial Sequence
  Fusion protein
MHVAQPAVVLASSRGIASFVCEYASPGKYTEVRVTVLRQADSQVTEVCAATYMMGNELTFLDDSICTGTSSGNQVNLTIQGLRAMDTGLYICKVELMYPPPYFEGIGNGTQIYVIDPEPCPDSDQEPKSSDKTHTSPPSPAPELLGGSSVFLFPPKPKDTLMISRTPEVTCVVVDVSHEDPEVKFNWYVDGVEVHNAKTKPREEQYNSTYRVVSVLTVLHQDWLNGKEYKCKVSNKALPAPIEKTISKAKGQPREPQVYTLPPSRDELTKNQVSLTCLVKGFYPSDIAVEWESNGQPENNYKTTPPVLDSDGSFFLYSKLTVDKSRWQQGNVFSCSVMHEALHNHYTQKSLSLSPGK

SEQ ID NO: 44 - protein, 357 aa, Artificial Sequence
  Fusion protein
MHVAQPAVVLASSRGIASFVCEYASPGKYTEVRVTVLRQADSQVTEVCAATYMMGNELTFLDDSICTGTSSGNQVNLTIQGLRAMDTGLYICKVELMYPPPYFDGIGNGTQIYVIDPEPCPDSDQEPKSSDKTHTSPPSPAPELLGGSSVFLFPPKPKDTLMISRTPEVTCVVVDVSHEDPEVKFNWYVDGVEVHNAKTKPREEQYNSTYRVVSVLTVLHQDWLNGKEYKCKVSNKALPAPIEKTISKAKGQPREPQVYTLPPSRDELTKNQVSLTCLVKGFYPSDIAVEWESNGQPENNYKTTPPVLDSDGSFFLYSKLTVDKSRWQQGNVFSCSVMHEALHNHYTQKSLSLSPGK

SEQ ID NO: 45 - protein, 357 aa, Artificial Sequence
  Fusion protein
MHVAQPAVVLASSRGIASFVCEYASPGKYTEVRVTVLRQADSQVTEVCAATYMMGNELTFLDDSICTGTSSGNQVNLTIQGLRAMDTGLYICKVELMYPPPYFVGIGNGTQIYVIDPEPCPDSDQEPKSSDKTHTSPPSPAPELLGGSSVFLFPPKPKDTLMISRTPEVTCVVVDVSHEDPEVKFNWYVDGVEVHNAKTKPREEQYNSTYRVVSVLTVLHQDWLNGKEYKCKVSNKALPAPIEKTISKAKGQPREPQVYTLPPSRDELTKNQVSLTCLVKGFYPSDIAVEWESNGQPENNYKTTPPVLDSDGSFFLYSKLTVDKSRWQQGNVFSCSVMHEALHNHYTQKSLSLSPGK

SEQ ID NO: 46 - protein, 124 aa, Artificial Sequence; identical to SEQ ID NO: 36
  Mutant

SEQ ID NO: 47 - protein, 124 aa, Artificial Sequence
  Mutant
MHVAQPAVVLASSRGIASFVCEYASPGKYTEVRVTVLRQADSQVTEVCAATYMMGNELTFLDDSICTGTSSGNQVNLTIQGLRAMDTGLYICKVELMYPPPYFEGIGNGTQIYVIDPEPCPDSD

SEQ ID NO: 48 - protein, 124 aa, Artificial Sequence
  Mutant
MHVAQPAVVLASSRGIASFVCEYASPGKYTEVRVTVLRQADSQVTEVCAATYMMGNELTFLDDSICTGTSSGNQVNLTIQGLRAMDTGLYICKVELMYPPPYFDGIGNGTQIYVIDPEPCPDSD

SEQ ID NO: 49 - protein, 124 aa, Artificial Sequence
  Mutant
MHVAQPAVVLASSRGIASFVCEYASPGKYTEVRVTVLRQADSQVTEVCAATYMMGNELTFLDDSICTGTSSGNQVNLTIQGLRAMDTGLYICKVELMYPPPYFVGIGNGTQIYVIDPEPCPDSD

SEQ ID NO: 50 - protein, 6 aa, Homo sapiens
MYPPPY